European Patent Specification EP 3 378 484 B1, published April 5, 2023. Title: Pharmaceutical Composition for Treating Cardiac Fibrosis. Applicant: BethphaGen Inc. The sequence listing filed with the application follows.

SEQUENCE LISTING (2 sequences)

SEQ ID NO: 1 - protein, 251 aa, Amino acid sequence of CCN5
MRGNPLIHLLAISFLCILSMVYAQLCPAPCACPWTPPQCPPGVPLVLDGCGCCRVCARRLGESCDHLHVCNPSQGLVCQPGAGPSGRGVVCLFEEDDGSCEVNGRRYLDGETFKPNCRVLCRCDDGGFTCLPLCSEDVRLPSWDCPRPRRIQVPGRCCPEWVCDQAVMQPAIQPSSAQGHQLSALVTPASADGPCPNWSTAWGPCSTTCGLGIATRVSNQNRFCQLEIQRRLCLSRPCLASRSHGSWNSAF

SEQ ID NO: 2 - DNA, 756 bp, Nucleotide sequence of CCN5
atgaggggcaacccactgatccatcttctggccatttccttcctctgcattctctcaatggtgtatgcccagctgtgcccagcaccctgtgcctgtccttggacaccaccccagtgcccaccgggggtacccctggtgctggatggctgtggctgctgtcgagtgtgtgcacggaggctgggggagtcctgcgaccacctgcatgtctgcaaccccagccagggcctggtttgtcagcctggggcaggccccagtggccgtggtgttgtgtgcctcttcgaagaggatgacgggagctgtgaggtgaacggccgcaggtacctggatggggagacctttaaacccaattgcagggttttgtgccgctgtgatgacggtggtttcacctgcctgccgctgtgcagtgaggatgtgcggctgcccagctgggactgcccacgccccaggagaatacaggtgccaggaaggtgctgccccgagtgggtgtgtgaccaggcagtgatgcagccggcaatccagccctcctcagcccaaggacaccaactttctgcccttgtcactcctgcatctgccgatggcccctgtccaaactggagcacagcctggggcccctgctcaaccacctgtgggttgggcatagccacccgagtatccaaccagaaccgattctgccaactggagatccagcgtcgcctgtgtctgtccagaccctgcctggcatccaggagccacggctcatggaacagtgccttctag